European Patent Specification EP 3 601 258 B1, published August 30, 2023. Title: COMPOUNDS USEFUL AS IMMUNOMODULATORS. Applicant: BRISTOL-MYERS SQUIBB COMPANY. The sequence listing filed with the application follows.

SEQUENCE LISTING (2 sequences)

SEQ ID NO: 1 - protein, 384 aa, Homo sapiens
LDSPDRPWNPPTFSPALLVVTEGDNATFTCSFSNTSESFVLNWYRMSPSNQTDKLAAFPEDRSQPGQDCRFRVTQLPNGRDFHMSVVRARRNDSGTYLCGAISLAPKAQIKESLRAELRVTERRAEVPTAHPSPSPRPAGQFQGSPGGGGGREPKSSDKTHTSPPSPAPELLGGSSVFLFPPKPKDTLMISRTPEVTCVVVDVSHEDPEVKFNWYVDGVEVHNAKTKPREEQYNSTYRVVSVLTVLHQDWLNGKEYKCKVSNKALPAPIEKTISKAKGQPREPQVYTLPPSRDELTKNQVSLTCLVKGFYPSDIAVEWESNGQPENNYKTTPPVLDSDGSFFLYSKLTVDKSRWQQGNVFSCSVMHEALHNHYTQKSLSLSPGK

SEQ ID NO: 2 - protein, 238 aa, Homo sapiens
AFTVTVPKDLYVVEYGSNMTIECKFPVEKQLDLAALIVYWEMEDKNIIQFVHGEEDLKVQHSSYRQRARLLKDQLSLGNAALQITDVKLQDAGVYRCMISYGGADYKRITVKVNAPYNKINQRILVVDPVTSEHELTCQAEGYPKAEVIWTSSDHQVLSGKTTTTNSKREEKLFNVTSTLRINTTTNEIFYCTFRRLDPEENHTAELVIPELPLAHPPNERTGSSETVRFQGHHHHHH